European Patent Application EP 4 141 120 A1, published March 1, 2023. Title: Production method for trimeric spike protein of Corona-19 virus in plants and its use for vaccination. Applicant: POSTECH ACADEMY-INDUSTRY FOUNDATION Korea Disease Control and Prevention Agency BioApplications Inc. The sequence listing filed with the application follows.

SEQUENCE LISTING (16 sequences)

SEQ ID NO: 1 - DNA, 3594 bp, Artificial Sequence
  Sf delta (TMD-CT)
gttaaccttaccaccagaactcagttacccccagcatacactaattctttcacacgtggtgtttactaccctgacaaagttttcagaagcagcgttttacacagcactcaggatttattcctacctttcttttccaacgtgacctggttccatgctatacatgtatctgggaccaatggtaccaagaggtttgataacccggtcctaccatttaatgatggagtctattttgcctccactgagaagtctaatataataagaggctggatttttggaactactcttgattcgaagacccagagtctacttattgttaataacgctacaaatgttgttatcaaagtatgtgaatttcaattctgtaatgatccattcttgggtgtttactaccacaaaaacaacaaaagttggatggaaagtgagtttcgggtttatagcagtgcgaataattgcacttttgagtacgtctcccaaccttttcttatggaccttgaaggaaagcagggaaatttcaagaatcttcgcgaatttgtgtttaagaatatcgatggttatttcaagatatattctaagcacacgcctattaatttagtgcgagatctccctcagggtttttcggcgctggaaccattggtagatttgccgataggaatcaatatcactaggttccagactttacttgctctgcatagaagttacttgacccctggagatagctcatcaggttggacagctggtgcggcagcttattacgtggggtatcttcagcctaggacgttcctattaaaatataatgaaaatggaaccattacagatgctgtagactgtgcacttgaccctctctcagaaacaaagtgtacgttgaaatccttcacggtagaaaaagggatctaccaaacgtctaacttcagagtccagccaacagaatctattgtgagatttcccaatattacaaacttgtgccctttcggagaagtttttaacgccaccaggtttgcatcggtttatgcttggaacaggaaaagaatcagcaactgtgttgctgattatagtgtcctatataactccgcatccttttccactttcaagtgttacggagtttctcctactaaattaaatgatctctgctttactaatgtctatgcagattcatttgtaatcagaggtgatgaggtcagacaaatcgctccagggcagactggaaagattgctgattataattataagcttcctgatgattttacaggctgcgttatagcatggaattctaataatcttgactctaaggtggggggaaattataattacctgtatagactgtttaggaagagcaatctcaagcctttcgagagagacatttcaactgagatctaccaggcgggaagcactccgtgtaatggtgttgagggttttaattgttactttcctttacagtcatacggtttccaacccacgaatggggttggttaccaaccgtaccgagtagtagtactttctttcgagcttctacatgccccagcaactgtttgtggacctaagaagtctactaatttggttaaaaataagtgtgtcaattttaatttcaatggacttacgggcacaggagttcttactgagtctaacaagaagtttctgcctttccagcagttcggcagagatattgctgacactactgatgctgtgcgtgatccacagacacttgaaattcttgacattacaccatgttcttttggtggcgtgagtgttataactcccggaacaaatacctccaaccaggtggctgttctgtatcaggacgtgaactgtacagaagtccctgttgcaattcatgcagatcagcttactcctacctggcgtgtttattctacgggttccaatgtttttcaaacacgtgcaggctgcttgataggggctgaacatgtcaacaactcatatgaatgcgacatacccataggtgcaggtatatgcgctagttatcagactcagaccaattctccgcggcgggcacgaagtgtagctagtcaatccatcattgcctacactatgtcacttggtgcagaaaattcagttgcttactctaataactctattgccatacccacaaattttactattagtgttaccacagaaattctaccagtgtctatgaccaagacatcagttgactgtacaatgtatatttgcggggattcaactgagtgctcgaatctgttgttgcaatacggcagtttttgtacccaattgaaccgggctctgactggaatagctgtggaacaagataaaaacacccaagaagtttttgcacaagtcaaacaaatttataaaacaccaccaattaaagatttcggtggtttcaacttctcacaaatactgccagatccgagcaaaccaagcaagaggtcattcattgaagacctacttttcaacaaagtgacacttgcagatgctggcttcattaaacagtatggtgattgcttgggggatattgctgctagagacctcatttgtgcacaaaagtttaacgggctgacagtgttgccacctttgttgacagatgagatgattgctcagtacacttctgcactgctcgctggtacaatcacatctgggtggacctttggtgcaggtgctgccttacaaataccatttgctatgcagatggcttataggttcaatggtatcggagttacacagaacgttctctatgagaaccaaaaattgattgccaaccaattcaatagtgccattggcaagattcaggactcactttcaagcacagcgagtgcacttggaaagttgcaagatgtggtcaaccagaatgcacaagctttaaacacgcttgtgaaacaactcagctccaactttggggcaatttcaagtgttttgaatgatatcctttcacgtcttgataaagtggaagccgaggtgcaaattgacaggttgatcacaggccgacttcaaagtttgcagacttatgtgactcaacaattaattagggcagcagaaatccgcgcttcggctaatctggcggctactaaaatgtcagagtgtgtacttggacaatctaaacgagttgatttttgcggaaagggctatcatctcatgtccttccctcagtcagcgcctcacggtgtagtgttcttgcacgtgacttacgttcctgcacaagaaaagaatttcacaactgctccggccatttgtcatgatggaaaagcccactttccgcgtgaaggtgtctttgtttcgaatggcacacactggtttgtaacccaaaggaatttttatgagccacaaatcattacgacggacaacacttttgtgtctggtaattgtgatgttgtaatcggaatcgtcaacaacaccgtttacgatcctttgcagcctgagttagattctttcaaagaggagctggataagtatttcaagaatcatacatcacccgatgttgatctcggtgatatctctggaattaatgcttcagttgtgaacattcaaaaggagattgaccgcctcaatgaggttgccaagaatttgaatgaatcgctcatcgatctccaagaacttggaaagtatgagcagtatatcaagtggcca

SEQ ID NO: 2 - protein, 1198 aa, Artificial Sequence
  Sf delta (TMD-CT)
VNLTTRTQLPPAYTNSFTRGVYYPDKVFRSSVLHSTQDLFLPFFSNVTWFHAIHVSGTNGTKRFDNPVLPFNDGVYFASTEKSNIIRGWIFGTTLDSKTQSLLIVNNATNVVIKVCEFQFCNDPFLGVYYHKNNKSWMESEFRVYSSANNCTFEYVSQPFLMDLEGKQGNFKNLREFVFKNIDGYFKIYSKHTPINLVRDLPQGFSALEPLVDLPIGINITRFQTLLALHRSYLTPGDSSSGWTAGAAAYYVGYLQPRTFLLKYNENGTITDAVDCALDPLSETKCTLKSFTVEKGIYQTSNFRVQPTESIVRFPNITNLCPFGEVFNATRFASVYAWNRKRISNCVADYSVLYNSASFSTFKCYGVSPTKLNDLCFTNVYADSFVIRGDEVRQIAPGQTGKIADYNYKLPDDFTGCVIAWNSNNLDSKVGGNYNYLYRLFRKSNLKPFERDISTEIYQAGSTPCNGVEGFNCYFPLQSYGFQPTNGVGYQPYRVVVLSFELLHAPATVCGPKKSTNLVKNKCVNFNFNGLTGTGVLTESNKKFLPFQQFGRDIADTTDAVRDPQTLEILDITPCSFGGVSVITPGTNTSNQVAVLYQDVNCTEVPVAIHADQLTPTWRVYSTGSNVFQTRAGCLIGAEHVNNSYECDIPIGAGICASYQTQTNSPRRARSVASQSIIAYTMSLGAENSVAYSNNSIAIPTNFTISVTTEILPVSMTKTSVDCTMYICGDSTECSNLLLQYGSFCTQLNRALTGIAVEQDKNTQEVFAQVKQIYKTPPIKDFGGFNFSQILPDPSKPSKRSFIEDLLFNKVTLADAGFIKQYGDCLGDIAARDLICAQKFNGLTVLPPLLTDEMIAQYTSALLAGTITSGWTFGAGAALQIPFAMQMAYRFNGIGVTQNVLYENQKLIANQFNSAIGKIQDSLSSTASALGKLQDVVNQNAQALNTLVKQLSSNFGAISSVLNDILSRLDKVEAEVQIDRLITGRLQSLQTYVTQQLIRAAEIRASANLAATKMSECVLGQSKRVDFCGKGYHLMSFPQSAPHGVVFLHVTYVPAQEKNFTTAPAICHDGKAHFPREGVFVSNGTHWFVTQRNFYEPQIITTDNTFVSGNCDVVIGIVNNTVYDPLQPELDSFKEELDKYFKNHTSPDVDLGDISGINASVVNIQKEIDRLNEVAKNLNESLIDLQELGKYEQYIKWP

SEQ ID NO: 3 - DNA, 1998 bp, Artificial Sequence
  S1s
gttaaccttaccaccagaactcagttacccccagcatacactaattctttcacacgtggtgtttactaccctgacaaagttttcagaagcagcgttttacacagcactcaggatttattcctacctttcttttccaacgtgacctggttccatgctatacatgtatctgggaccaatggtaccaagaggtttgataacccggtcctaccatttaatgatggagtctattttgcctccactgagaagtctaatataataagaggctggatttttggaactactcttgattcgaagacccagagtctacttattgttaataacgctacaaatgttgttatcaaagtatgtgaatttcaattctgtaatgatccattcttgggtgtttactaccacaaaaacaacaaaagttggatggaaagtgagtttcgggtttatagcagtgcgaataattgcacttttgagtacgtctcccaaccttttcttatggaccttgaaggaaagcagggaaatttcaagaatcttcgcgaatttgtgtttaagaatatcgatggttatttcaagatatattctaagcacacgcctattaatttagtgcgagatctccctcagggtttttcggcgctggaaccattggtagatttgccgataggaatcaatatcactaggttccagactttacttgctctgcatagaagttacttgacccctggagatagctcatcaggttggacagctggtgcggcagcttattacgtggggtatcttcagcctaggacgttcctattaaaatataatgaaaatggaaccattacagatgctgtagactgtgcacttgaccctctctcagaaacaaagtgtacgttgaaatccttcacggtagaaaaagggatctaccaaacgtctaacttcagagtccagccaacagaatctattgtgagatttcccaatattacaaacttgtgccctttcggagaagtttttaacgccaccaggtttgcatcggtttatgcttggaacaggaaaagaatcagcaactgtgttgctgattatagtgtcctatataactccgcatccttttccactttcaagtgttacggagtttctcctactaaattaaatgatctctgctttactaatgtctatgcagattcatttgtaatcagaggtgatgaggtcagacaaatcgctccagggcagactggaaagattgctgattataattataagcttcctgatgattttacaggctgcgttatagcatggaattctaataatcttgactctaaggtggggggaaattataattacctgtatagactgtttaggaagagcaatctcaagcctttcgagagagacatttcaactgagatctaccaggcgggaagcactccgtgtaatggtgttgagggttttaattgttactttcctttacagtcatacggtttccaacccacgaatggggttggttaccaaccgtaccgagtagtagtactttctttcgagcttctacatgccccagcaactgtttgtggacctaagaagtctactaatttggttaaaaataagtgtgtcaattttaatttcaatggacttacgggcacaggagttcttactgagtctaacaagaagtttctgcctttccagcagttcggcagagatattgctgacactactgatgctgtgcgtgatccacagacacttgaaattcttgacattacaccatgttcttttggtggcgtgagtgttataactcccggaacaaatacctccaaccaggtggctgttctgtatcaggacgtgaactgtacagaagtccctgttgcaattcatgcagatcagcttactcctacctggcgtgtttattctacgggttccaatgtttttcaaacacgtgcaggctgcttgataggggctgaacatgtcaacaactcatatgaatgcgacatacccataggtgcaggtatatgcgctagttatcagactcagaccaattctccg

SEQ ID NO: 4 - protein, 666 aa, Artificial Sequence
  S1s protein
VNLTTRTQLPPAYTNSFTRGVYYPDKVFRSSVLHSTQDLFLPFFSNVTWFHAIHVSGTNGTKRFDNPVLPFNDGVYFASTEKSNIIRGWIFGTTLDSKTQSLLIVNNATNVVIKVCEFQFCNDPFLGVYYHKNNKSWMESEFRVYSSANNCTFEYVSQPFLMDLEGKQGNFKNLREFVFKNIDGYFKIYSKHTPINLVRDLPQGFSALEPLVDLPIGINITRFQTLLALHRSYLTPGDSSSGWTAGAAAYYVGYLQPRTFLLKYNENGTITDAVDCALDPLSETKCTLKSFTVEKGIYQTSNFRVQPTESIVRFPNITNLCPFGEVFNATRFASVYAWNRKRISNCVADYSVLYNSASFSTFKCYGVSPTKLNDLCFTNVYADSFVIRGDEVRQIAPGQTGKIADYNYKLPDDFTGCVIAWNSNNLDSKVGGNYNYLYRLFRKSNLKPFERDISTEIYQAGSTPCNGVEGFNCYFPLQSYGFQPTNGVGYQPYRVVVLSFELLHAPATVCGPKKSTNLVKNKCVNFNFNGLTGTGVLTESNKKFLPFQQFGRDIADTTDAVRDPQTLEILDITPCSFGGVSVITPGTNTSNQVAVLYQDVNCTEVPVAIHADQLTPTWRVYSTGSNVFQTRAGCLIGAEHVNNSYECDIPIGAGICASYQTQTNSP

SEQ ID NO: 5 - DNA, 1596 bp, Artificial Sequence
  S2s delta (TMD-CT)
cggcgggcacgaagtgtagctagtcaatccatcattgcctacactatgtcacttggtgcagaaaattcagttgcttactctaataactctattgccatacccacaaattttactattagtgttaccacagaaattctaccagtgtctatgaccaagacatcagttgactgtacaatgtatatttgcggggattcaactgagtgctcgaatctgttgttgcaatacggcagtttttgtacccaattgaaccgggctctgactggaatagctgtggaacaagataaaaacacccaagaagtttttgcacaagtcaaacaaatttataaaacaccaccaattaaagatttcggtggtttcaacttctcacaaatactgccagatccgagcaaaccaagcaagaggtcattcattgaagacctacttttcaacaaagtgacacttgcagatgctggcttcattaaacagtatggtgattgcttgggggatattgctgctagagacctcatttgtgcacaaaagtttaacgggctgacagtgttgccacctttgttgacagatgagatgattgctcagtacacttctgcactgctcgctggtacaatcacatctgggtggacctttggtgcaggtgctgccttacaaataccatttgctatgcagatggcttataggttcaatggtatcggagttacacagaacgttctctatgagaaccaaaaattgattgccaaccaattcaatagtgccattggcaagattcaggactcactttcaagcacagcgagtgcacttggaaagttgcaagatgtggtcaaccagaatgcacaagctttaaacacgcttgtgaaacaactcagctccaactttggggcaatttcaagtgttttgaatgatatcctttcacgtcttgataaagtggaagccgaggtgcaaattgacaggttgatcacaggccgacttcaaagtttgcagacttatgtgactcaacaattaattagggcagcagaaatccgcgcttcggctaatctggcggctactaaaatgtcagagtgtgtacttggacaatctaaacgagttgatttttgcggaaagggctatcatctcatgtccttccctcagtcagcgcctcacggtgtagtgttcttgcacgtgacttacgttcctgcacaagaaaagaatttcacaactgctccggccatttgtcatgatggaaaagcccactttccgcgtgaaggtgtctttgtttcgaatggcacacactggtttgtaacccaaaggaatttttatgagccacaaatcattacgacggacaacacttttgtgtctggtaattgtgatgttgtaatcggaatcgtcaacaacaccgtttacgatcctttgcagcctgagttagattctttcaaagaggagctggataagtatttcaagaatcatacatcacccgatgttgatctcggtgatatctctggaattaatgcttcagttgtgaacattcaaaaggagattgaccgcctcaatgaggttgccaagaatttgaatgaatcgctcatcgatctccaagaacttggaaagtatgagcagtatatcaagtggcca

SEQ ID NO: 6 - protein, 532 aa, Artificial Sequence
  S2s delta (TMD-CT)
RRARSVASQSIIAYTMSLGAENSVAYSNNSIAIPTNFTISVTTEILPVSMTKTSVDCTMYICGDSTECSNLLLQYGSFCTQLNRALTGIAVEQDKNTQEVFAQVKQIYKTPPIKDFGGFNFSQILPDPSKPSKRSFIEDLLFNKVTLADAGFIKQYGDCLGDIAARDLICAQKFNGLTVLPPLLTDEMIAQYTSALLAGTITSGWTFGAGAALQIPFAMQMAYRFNGIGVTQNVLYENQKLIANQFNSAIGKIQDSLSSTASALGKLQDVVNQNAQALNTLVKQLSSNFGAISSVLNDILSRLDKVEAEVQIDRLITGRLQSLQTYVTQQLIRAAEIRASANLAATKMSECVLGQSKRVDFCGKGYHLMSFPQSAPHGVVFLHVTYVPAQEKNFTTAPAICHDGKAHFPREGVFVSNGTHWFVTQRNFYEPQIITTDNTFVSGNCDVVIGIVNNTVYDPLQPELDSFKEELDKYFKNHTSPDVDLGDISGINASVVNIQKEIDRLNEVAKNLNESLIDLQELGKYEQYIKWP

SEQ ID NO: 7 - DNA, 96 bp, Artificial Sequence
  mCOr1
gtgtctaggcttgaggaagatgttagaaatctcaacgcaattgtccagaaacttcaggaaaggttggataggctggaggaaactgttcaagctaag

SEQ ID NO: 8 - protein, 32 aa, Artificial Sequence
  mCor1
VSRLEEDVRNLNAIVQKLQERLDRLEETVQAK

SEQ ID NO: 9 - DNA, 36 bp, Artificial Sequence
  Linker
ggaggttcaggaggttcaggaggttcaggaggttca

SEQ ID NO: 10 - protein, 12 aa, Artificial Sequence
  Linker
GGSGGSGGSGGS

SEQ ID NO: 11 - DNA, 272 bp, Artificial Sequence
  BiP
atggctcgctcgtttggagctaacagtaccgttgtgttggcgatcatcttcttcggtgagtgattttccgatcttcttctccgatttagatctcctctacattgttgcttaatctcagaaccttttttcgttgttcctggatctgaatgtgtttgtttgcaatttcacgatcttaaaaggttagatctcgattggtattgacgattggaatctttacgatttcaggatgtttatttgcgttgtcctctgcaatagaagaggctacgaagtta

SEQ ID NO: 12 - DNA, 12 bp, Artificial Sequence
  HDEL
cacgatgagctc

SEQ ID NO: 13 - protein, 4 aa, Artificial Sequence
  HDEL
HDEL

SEQ ID NO: 14 - DNA, 22 bp, Artificial Sequence
  5'UTR
aattattacatcaaaacaaaaa

SEQ ID NO: 15 - DNA, 1220 bp, Artificial Sequence
  MacT
agagatctcctttgccccagagatcacaatggacgacttcctctatctctacgatctagtcaggaagttcgacggagaaggtgacgataccatgttcaccactgataatgagaagattagccttttcaatttcagaaagaatgctaacccacagatggttagagaggcttacgcagcaggtctcatcaagacgatctacccgagcaataatctccaggagatcaaataccttcccaagaaggttaaagatgcagtcaaaagattcaggactaactgcatcaagaacacagagaaagatatatttctcaagatcagaagtactattccagtatggacgattcaaggcttgcttcacaaaccaaggcaagtaatagagattggagtctctaaaaaggtagttcccactgaatcaaaggccatggagtcaaagattcaaatagaggacctaacagaactcgccgtaaagactggcgaacagttcatacagagtctcttacgactcaatgacaagaagaaaatcttcgtcaacatggtggagcacgacacgcttgtctactccaaaaatatcaaagatacagtctcagaagaccaaagggcaattgagacttttcaacaaagggtaatatccggaaacctcctcggattccattgcccagctatctgtcactttattgtgaagatagtggaaaaggaaggtggctcctacaaatgccatcattgcgataaaggaaaggccatcgttgaagatgcctctgccgacagtggtcccaaagatggacccccacccacgaggagcatcgtggaaaaagaagacgttccaaccacgtcttcaaagcaagtggattgatgtgacgcaagacgtgacgtaagtatctgagctagtttttatttttctactaatttggtcgtttatttcggcgtgtaggacatggcaaccgggcctgaatttcgcgggtattctgtttctattccaactttttcttgatccgcagccattaacgacttttgaatagatacgctgacacgccaagcctcgctagtcaaaagtgtaccaaacaacgctttacagcaagaacggaatgcgcgtgacgctcgcggtgacgccatttcgccttttcagaaatggataaatagccttgcttcctattatatcttcccaaattaccaatacattacactagcatctgaatttcataaccaatctcgatacaccaaatcgt

SEQ ID NO: 16 - DNA, 520 bp, Artificial Sequence
  RD29B terminator
aattttactcaaaatgttttggttgctatggtagggactatggggttttcggattccggtggaagtgagtggggaggcagtggcggaggtaagggagttcaagattctggaactgaagatttggggttttgcttttgaatgtttgcgtttttgtatgatgcctctgtttgtgaactttgatgtattttatctttgtgtgaaaaagagattgggttaataaaatatttgcttttttggataagaaactcttttagcggcccattaataaaggttacaaatgcaaaatcatgttagcgtcagatatttaattattcgaagatgattgtgatagatttaaaattatcctagtcaaaaagaaagagtaggttgagcagaaacagtgacatctgttgtttgtaccatacaaattagtttagattattggttaacatgttaaatggctatgcatgtgacatttagaccttatcggaattaatttgtagaattattaattaagatgttgattagttcaaacaaaaat